European Patent Application EP 4 342 909 A1, published March 27, 2024. Title: Anti-norovirus antibody. Applicant: DENKA COMPANY LIMITED. The sequence listing filed with the application follows.

SEQUENCE LISTING (3 sequences)

SEQ ID NO: 1 - protein, 23 aa, Artificial Sequence
  partial sequence of shell domain of capsid of norovirus
MLYTPLRTGGGSGGTDPFVVAGR

SEQ ID NO: 2 - protein, 23 aa, Artificial Sequence
  partial sequence of shell domain of capsid of norovirus
RLVAMLYTPLRANGSGDDVFTVS

SEQ ID NO: 3 - protein, 7 aa, Artificial Sequence
  partial sequence of shell domain of capsid of norovirus
MLYTPLR